European Patent Specification EP 3 801 465 B1, published July 24, 2024. Title: DEMETHYLATION TO TREAT EYE DISEASE. Applicant: THE REGENTS OF THE UNIVERSITY OF CALIFORNIA. The sequence listing filed with the application follows.

SEQUENCE LISTING (32 sequences)

SEQ ID NO: 1 - DNA, 20 bp, Artificial Sequence
  Description of Artificial Sequence: Synthetic primer
gtaattccgtgatcaccgtc

SEQ ID NO: 2 - DNA, 20 bp, Artificial Sequence
  Description of Artificial Sequence: Synthetic primer
ccaataaataacagcagaag

SEQ ID NO: 3 - DNA, 20 bp, Artificial Sequence
  Description of Artificial Sequence: Synthetic primer
caatatgctcatcattgtct

SEQ ID NO: 4 - DNA, 20 bp, Artificial Sequence
  Description of Artificial Sequence: Synthetic primer
ccacacatgtctaccttcct

SEQ ID NO: 5 - DNA, 19 bp, Artificial Sequence
  Description of Artificial Sequence: Synthetic primer
cgatttgcaggtccagccg

SEQ ID NO: 6 - DNA, 19 bp, Artificial Sequence
  Description of Artificial Sequence: Synthetic primer
cagcgggtgggtattcctg

SEQ ID NO: 7 - DNA, 20 bp, Artificial Sequence
  Description of Artificial Sequence: Synthetic primer
ctaggtgtggacatctcttg

SEQ ID NO: 8 - DNA, 17 bp, Artificial Sequence
  Description of Artificial Sequence: Synthetic primer
tgcaggagcgtacagaa

SEQ ID NO: 9 - DNA, 16 bp, Artificial Sequence
  Description of Artificial Sequence: Synthetic primer
agctcctccgctactc

SEQ ID NO: 10 - DNA, 16 bp, Artificial Sequence
  Description of Artificial Sequence: Synthetic primer
ccagcccttggtcatc

SEQ ID NO: 11 - DNA, 20 bp, Artificial Sequence
  Description of Artificial Sequence: Synthetic primer
taggcccagatgtacaggaa

SEQ ID NO: 12 - DNA, 20 bp, Artificial Sequence
  Description of Artificial Sequence: Synthetic primer
ccagaatgcaggcctagtaa

SEQ ID NO: 13 - DNA, 20 bp, Artificial Sequence
  Description of Artificial Sequence: Synthetic primer
gcggatcatggaacatctaa

SEQ ID NO: 14 - DNA, 20 bp, Artificial Sequence
  Description of Artificial Sequence: Synthetic primer
ccagccatattgagagcaga

SEQ ID NO: 15 - DNA, 22 bp, Artificial Sequence
  Description of Artificial Sequence: Synthetic primer
caccattggcaatgagcggttc

SEQ ID NO: 16 - DNA, 22 bp, Artificial Sequence
  Description of Artificial Sequence: Synthetic primer
aggtctttgcggatgtccacgt

SEQ ID NO: 17 - protein, 17 aa, Artificial Sequence
  Description of Artificial Sequence: Synthetic peptide
FPFGCLIFQSSYMMTLV

SEQ ID NO: 18 - DNA, 51 bp, Artificial Sequence
  Description of Artificial Sequence: Synthetic oligonucleotide
ttcccctttggctgtctcatcttccagtcttcctatatgatgacgctggtc

SEQ ID NO: 19 - DNA, 51 bp, Artificial Sequence
  Description of Artificial Sequence: Synthetic oligonucleotide
tttcccttcggctggctcatcttccagtcttcctatatgatgacgttagtc

SEQ ID NO: 20 - protein, 17 aa, Artificial Sequence
  Description of Artificial Sequence: Synthetic peptide
FPFGWLIFQSSYMMTLV

SEQ ID NO: 21 - protein, 299 aa, Homo sapiens
MEHFDASLSTYFKALLGPRDTRVKGWFLLDNYIPTFICSVIYLLIVWLGPKYMRNKQPFSCRGILVVYNLGLTLLSLYMFCELVTGVWEGKYNFFCQGTRTAGESDMKIIRVLWWYYFSKLIEFMDTFFFILRKNNHQITVLHVYHHASMLNIWWFVMNWVPCGHSYFGATLNSFIHVLMYSYYGLSSVPSMRPYLWWKKYITQGQLLQFVLTIIQTSCGVIWPCTFPLGWLYFQIGYMISLIALFTNFYIQTYNKKGASRRKDHLKDHQNGSMAAVNGHTNSFSPLENNVKPRKLRKD

SEQ ID NO: 22 - protein, 299 aa, Mus sp.
MEHFDASLSTYFKAFLGPRDTRVKGWFLLDNYIPTFVCSVIYLLIVWLGPKYMKNRQPFSCRGILQLYNLGLTLLSLYMFYELVTGVWEGKYNFFCQGTRSAGESDMKIIRVLWWYYFSKLIEFMDTFFFILRKNNHQITVLHVYHHATMLNIWWFVMNWVPCGHSYFGATLNSFIHVLMYSYYGLSSIPSMRPYLWWKKYITQGQLVQFVLTIIQTTCGVFWPCSFPLGWLFFQIGYMISLIALFTNFYIQTYNKKGASRRKDHLKGHQNGSVAAVNGHTNSFPSLENSVKPRKQRKD

SEQ ID NO: 23 - protein, 296 aa, Homo sapiens
MEHLKAFDDEINAFLDNMFGPRDSRVRGWFMLDSYLPTFFLTVMYLLSIWLGNKYMKNRPALSLRGILTLYNLGITLLSAYMLAELILSTWEGGYNLQCQDLTSAGEADIRVAKVLWWYYFSKSVEFLDTIFFVLRKKTSQITFLHVYHHASMFNIWWCVLNWIPCGQSFFGPTLNSFIHILMYSYYGLSVFPSMHKYLWWKKYLTQAQLVQFVLTITHTMSAVVKPCGFPFGCLIFQSSYMLTLVILFLNFYVQTYRKKPMKKDMQEPPAGKEVKNGFSKAYFTAANGVMNKKAQ

SEQ ID NO: 24 - protein, 292 aa, Mus sp.
MEQLKAFDNEVNAFLDNMFGPRDSRVRGWFLLDSYLPTFILTITYLLSIWLGNKYMKNRPALSLRGILTLYNLAITLLSAYMLVELILSSWEGGYNLQCQNLDSAGEGDVRVAKVLWWYYFSKLVEFLDTIFFVLRKKTNQITFLHVYHHASMFNIWWCVLNWIPCGQSFFGPTLNSFIHILMYSYYGLSVFPSMHKYLWWKKYLTQAQLVQFVLTITHTLSAVVKPCGFPFGCLIFQSSYMMTLVILFLNFYIQTYRKKPVKKELQEKEVKNGFPKAHLIVANGMTDKKAQ

SEQ ID NO: 25 - DNA, 194 bp, Artificial Sequence
  Description of Artificial Sequence: Synthetic polynucleotide
tgccttccaggtgcagttcgtactcaccatcacgcacacgctgagtgccgtggtgaagccctgtggctttcccttcggctggctcatcttccagtcttcctatatgatgacgttagtcatcctgttcttaaacttctatattcaggtaagtaagatgtgagtgttcaggggcaggcaacatatcagacagccca

SEQ ID NO: 26 - protein, 17 aa, Mus sp.
FPFGCLIFQSSYMMTLV

SEQ ID NO: 27 - DNA, 51 bp, Mus sp.
gaccagcgtcatcatataggaagactggaagatgagacagccaaaggggaa

SEQ ID NO: 28 - DNA, 51 bp, Mus sp.
gactaacgtcatcatataggaagactggaagatgagccagccgaagggaaa

SEQ ID NO: 29 - protein, 17 aa, Mus sp.
FPFGWLIFQSSYMMTLV

SEQ ID NO: 30 - DNA, 23 bp, Artificial Sequence
  Description of Artificial Sequence: Synthetic oligonucleotide
  modified_base (21)..(21): a, c, t, g, unknown or other
gtcttcctatatgatgacgcngg

SEQ ID NO: 31 - DNA, 25 bp, Artificial Sequence
  Description of Artificial Sequence: Synthetic oligonucleotide
gtctcccttgatatgatgaagcagg

SEQ ID NO: 32 - DNA, 24 bp, Artificial Sequence
  Description of Artificial Sequence: Synthetic oligonucleotide
gtcttcctaaatgatgcaggcagg